European Patent Specification EP 3 486 650 B1, published March 12, 2025. Title: Method for determining efficacy of removing virus during purification. Applicant: KWR Water B.V. The sequence listing filed with the application follows.

SEQUENCE LISTING (84 sequences)

SEQ ID NO: 1 - DNA, 20 bp, Artificial Sequence
  primer
accaggggcggtgtatattg

SEQ ID NO: 2 - DNA, 20 bp, Artificial Sequence
  primer
gccataattggcttcagcgg

SEQ ID NO: 3 - DNA, 20 bp, Artificial Sequence
  primer
ttacgccagccaaggtgaat

SEQ ID NO: 4 - DNA, 20 bp, Artificial Sequence
  primer
ttacgccagccaaggtgaat

SEQ ID NO: 5 - DNA, 20 bp, Artificial Sequence
  primer
accgaaacaccaaaccacct

SEQ ID NO: 6 - DNA, 20 bp, Artificial Sequence
  primer
tgttccggtagctttctgcc

SEQ ID NO: 7 - DNA, 20 bp, Artificial Sequence
  primer
gcatcttcgtcaatgcgtcc

SEQ ID NO: 8 - DNA, 20 bp, Artificial Sequence
  primer
tggactccaacgctcacatc

SEQ ID NO: 9 - DNA, 20 bp, Artificial Sequence
  primer
gcgatgaccgctcatttgtc

SEQ ID NO: 10 - DNA, 20 bp, Artificial Sequence
  primer
acctcgtggtagagacccaa

SEQ ID NO: 11 - DNA, 20 bp, Artificial Sequence
  primer
gacgccgttgaaatgtcagg

SEQ ID NO: 12 - DNA, 20 bp, Artificial Sequence
  primer
tcgcgcacttggtcaaaaag

SEQ ID NO: 13 - DNA, 20 bp, Artificial Sequence
  primer
atctttcaagccgcccatga

SEQ ID NO: 14 - DNA, 20 bp, Artificial Sequence
  primer
tctagttgctgccgttggag

SEQ ID NO: 15 - DNA, 20 bp, Artificial Sequence
  primer
accgcatagaatccagcgag

SEQ ID NO: 16 - DNA, 20 bp, Artificial Sequence
  primer
atcgggattcagtatggggc

SEQ ID NO: 17 - DNA, 20 bp, Artificial Sequence
  primer
gaggtcgtggtgtggctatc

SEQ ID NO: 18 - DNA, 20 bp, Artificial Sequence
  primer
cgttatttcagcgtcctgcg

SEQ ID NO: 19 - DNA, 20 bp, Artificial Sequence
  primer
cgctgtctgctgtgagtgta

SEQ ID NO: 20 - DNA, 20 bp, Artificial Sequence
  primer
catcggggtgtctgcttgat

SEQ ID NO: 21 - DNA, 20 bp, Artificial Sequence
  primer
tgtcggagcgtttccaatga

SEQ ID NO: 22 - DNA, 20 bp, Artificial Sequence
  primer
ttaaagatgccttgcccggt

SEQ ID NO: 23 - DNA, 20 bp, Artificial Sequence
  primer
tggtaaccgtgaacatcccg

SEQ ID NO: 24 - DNA, 20 bp, Artificial Sequence
  primer
ttgttcgactaatccggccc

SEQ ID NO: 25 - DNA, 20 bp, Artificial Sequence
  primer
cgagaagacactcggactcg

SEQ ID NO: 26 - DNA, 20 bp, Artificial Sequence
  primer
tgccccatactgaatcccga

SEQ ID NO: 27 - DNA, 20 bp, Artificial Sequence
  primer
ttgagaagcgagccgagaag

SEQ ID NO: 28 - DNA, 20 bp, Artificial Sequence
  primer
cgccatgtgggcaaaaatga

SEQ ID NO: 29 - DNA, 20 bp, Artificial Sequence
  primer
gggcgaaactaccaaccaga

SEQ ID NO: 30 - DNA, 20 bp, Artificial Sequence
  primer
gccttacaccggttggagaa

SEQ ID NO: 31 - DNA, 20 bp, Artificial Sequence
  primer
ttgtcaacccacgttggagc

SEQ ID NO: 32 - DNA, 20 bp, Artificial Sequence
  primer
gcattcgggaaagcggaatc

SEQ ID NO: 33 - DNA, 20 bp, Artificial Sequence
  primer
actgctgatcgcaatcccaa

SEQ ID NO: 34 - DNA, 20 bp, Artificial Sequence
  primer
cccattgtcgtcaacggaga

SEQ ID NO: 35 - DNA, 20 bp, Artificial Sequence
  primer
cgcatctgaagccgctaaac

SEQ ID NO: 36 - DNA, 22 bp, Artificial Sequence
  primer
tcggagcaacatcagcaataga

SEQ ID NO: 37 - DNA, 20 bp, Artificial Sequence
  primer
ggatagcgtctcgtcgatgg

SEQ ID NO: 38 - DNA, 20 bp, Artificial Sequence
  primer
cgcttaaatcctgcgaaccg

SEQ ID NO: 39 - DNA, 20 bp, Artificial Sequence
  primer
gtatggtagcgatgccgtga

SEQ ID NO: 40 - DNA, 20 bp, Artificial Sequence
  primer
cggtcagctggtaaggttcc

SEQ ID NO: 41 - DNA, 20 bp, Artificial Sequence
  primer
tgttgaaaaaggtgctgcgg

SEQ ID NO: 42 - DNA, 20 bp, Artificial Sequence
  primer
ttgtccacccgtgctcatac

SEQ ID NO: 43 - DNA, 20 bp, Artificial Sequence
  primer
actagccatttctgcccacc

SEQ ID NO: 44 - DNA, 20 bp, Artificial Sequence
  primer
ccaaacaaggttgctaccgc

SEQ ID NO: 45 - DNA, 20 bp, Artificial Sequence
  primer
gcaaaggatagctcgcaacg

SEQ ID NO: 46 - DNA, 20 bp, Artificial Sequence
  primer
tgttgcgatccttccagtcc

SEQ ID NO: 47 - DNA, 20 bp, Artificial Sequence
  primer
gtactgacgtgtcagctggt

SEQ ID NO: 48 - DNA, 20 bp, Artificial Sequence
  primer
ctatcgcaaaccgcaagagc

SEQ ID NO: 49 - DNA, 20 bp, Artificial Sequence
  primer
tgctcggaggttgagatgtg

SEQ ID NO: 50 - DNA, 20 bp, Artificial Sequence
  primer
tgagtcatcccccatggcta

SEQ ID NO: 51 - DNA, 20 bp, Artificial Sequence
  primer
gacatgcggcatccatcaac

SEQ ID NO: 52 - DNA, 20 bp, Artificial Sequence
  primer
gactgcccttgctcagaagt

SEQ ID NO: 53 - DNA, 20 bp, Artificial Sequence
  primer
ctacagcgtctcctgcgaat

SEQ ID NO: 54 - DNA, 20 bp, Artificial Sequence
  primer
agcagttttggactcgcgta

SEQ ID NO: 55 - DNA, 20 bp, Artificial Sequence
  primer
tacgctcgtatgctcgtcac

SEQ ID NO: 56 - DNA, 20 bp, Artificial Sequence
  primer
tggcaggaagtggtcgattc

SEQ ID NO: 57 - DNA, 20 bp, Artificial Sequence
  primer
agcgatgatgtggatgccaa

SEQ ID NO: 58 - DNA, 20 bp, Artificial Sequence
  primer
acctgcgtcttgggttactg

SEQ ID NO: 59 - DNA, 20 bp, Artificial Sequence
  primer
caaacatggtcgcgtgatga

SEQ ID NO: 60 - DNA, 20 bp, Artificial Sequence
  primer
taaggtgagcgttcgagcag

SEQ ID NO: 61 - DNA, 20 bp, Artificial Sequence
  primer
aggctcgtacctaacgtcct

SEQ ID NO: 62 - DNA, 20 bp, Artificial Sequence
  primer
ccgaaatgctgaccatgcag

SEQ ID NO: 63 - DNA, 20 bp, Artificial Sequence
  primer
agcgttggagaattcgtggt

SEQ ID NO: 64 - DNA, 20 bp, Artificial Sequence
  primer
ctcaaatcggttctggccct

SEQ ID NO: 65 - DNA, 20 bp, Artificial Sequence
  primer
atgcgttgccattttcccac

SEQ ID NO: 66 - DNA, 20 bp, Artificial Sequence
  primer
agggatcgttcagccacaag

SEQ ID NO: 67 - DNA, 20 bp, Artificial Sequence
  primer
atagaatgtactggccgccg

SEQ ID NO: 68 - DNA, 20 bp, Artificial Sequence
  primer
acgggaacacttgcatcctt

SEQ ID NO: 69 - DNA, 20 bp, Artificial Sequence
  primer
ctgccgtccagtttggtttg

SEQ ID NO: 70 - DNA, 20 bp, Artificial Sequence
  primer
aagtatgccccaggtcgttg

SEQ ID NO: 71 - DNA, 20 bp, Artificial Sequence
  primer
gagccgttggcagacttaca

SEQ ID NO: 72 - DNA, 20 bp, Artificial Sequence
  primer
cgcactaagaagggtgcaga

SEQ ID NO: 73 - DNA, 20 bp, Artificial Sequence
  primer
gtctgaaacgcgattggtgg

SEQ ID NO: 74 - DNA, 20 bp, Artificial Sequence
  primer
gtgctgcctcctaacggaat

SEQ ID NO: 75 - DNA, 20 bp, Artificial Sequence
  primer
ccgcaagccttgatggaaag

SEQ ID NO: 76 - DNA, 20 bp, Artificial Sequence
  primer
cctggcaagattagcgtcca

SEQ ID NO: 77 - DNA, 20 bp, Artificial Sequence
  primer
atgtgcagtcgtggattcgt

SEQ ID NO: 78 - DNA, 20 bp, Artificial Sequence
  primer
gtggagctccgaggtattcg

SEQ ID NO: 79 - DNA, 20 bp, Artificial Sequence
  primer
gttacacgccgacaccaaac

SEQ ID NO: 80 - DNA, 20 bp, Artificial Sequence
  primer
gagcggacgcacaatttgat

SEQ ID NO: 81 - DNA, 20 bp, Artificial Sequence
  primer
actggcaggtgcacatagta

SEQ ID NO: 82 - DNA, 20 bp, Artificial Sequence
  primer
ctggttccggatcggacttc

SEQ ID NO: 83 - DNA, 20 bp, Artificial Sequence
  primer
agggtccatctgtcctcgaa

SEQ ID NO: 84 - DNA, 20 bp, Artificial Sequence
  primer
tgaccattatcccgctcacg